European Patent Application EP 4 686 480 A1, published February 4, 2026. Title: Live Attenuated E. Coli Vaccine. Applicant: Institut fur Virologie und Immunologie (IVI). Application EP. The sequence listing filed with the application follows.

SEQUENCE LISTING (5 sequences)

SEQ ID NO: 1 - DNA, 1080 bp, Escherichia coli
  source 1..1080: mol_type = genomic DNA
atgcaagcggcaactgttgtgattaaccgccgcgctctgcgacacaacctgcaacgtcttcgtgaactggcgcctgccagtaaaatggttgcggtggtgaaagcgaacgcttatggtcacggtcttcttgagaccgcgcgaacgctccccgatgctgacgcctttggcgtagcccgtctcgaagaagctctgcgactgcgtgcggggggaatcaccaaacctgtacttttactcgaaggcttttttgatgccagagatctaccgacgatttctgcgcaacattttcataccgccgtgcataacgaagaacagctggctgcgctggaagaggctagcctggacgagccggttaccgtctggatgaaactcgataccggtatgcaccgtctgggcgtaaggccggaacaggctgaggcgttttatcatcgtctgacccagtgcaaaaacgttcgtcagccggtgaatatcgtcagccattttgcgcgcgcggatgaaccaaaatgcggcgcaaccgagaagcaactcgctatctttaataccttttgcgaaggcaaacctggtcaacgttccattgccgcgtcgggtggcattttactctggccacagtcgcattttgactgggtgcgcccgggcatcattctttacggcgtatctccgctggaagatcgctccaccggtgccgattttggctgtcagccagtgatgtcgctaacctccagcctgattgccgtgcgtgagcataaagccggagagcctgtcggttatggtggaacctgggtaagcgaacgtgatactcgtcttggcgtagtcgcgatgggctatggcgatggttatccgcgcgccgcgccgtccggtacgccagtgctggtgaacggtcgcgaagtgccgattgtcgggcgcgtggcgatggatatgatctgcgtagacttaggtccacaggcgcaggataaagccggggacccggtcattttatggggcgaaggtttgcccgtagaacgtatcgctgaaatgacgaaagtaagtgcttacgaacttatcacgcgcctgacctcaagagtcgcgatgaaatacgtggattaa

SEQ ID NO: 2 - DNA, 1104 bp, Escherichia coli
  source 1..1104: mol_type = genomic DNA
ttacgccagttgacgaagcatccgacgcagcggctccgcggccccccacagcagctggtcgcccacggtaaaggctgacaggaactccggtcccatattcagcttacgcaggcggcctaccggcgtggtcagcgtgccggtaacggcagctggggttagctcacgcatagtgatttcccgatcgttcggaacaactttcgcccacggattgtgcgcagccagcagttcttccacggtcggaatagacacatcttttttcaatttaatagtgaatgcctggctgtggcagcgcaatgccccgacacgcacacataaaccatctaccggaattacggaagatgtgttgaggatcttgttggtttccgcctgccctttccactcttcgcggctctgaccgttatcaagctgtttgtcgatccacggaatcaggctacccgccagcggcacgccaaagttatctaccggcagctcaccgctacgggttaaggttgtgactttgcgttcgatatcgagaatagcagaggacgggttcgcgagttcatctgccacatggccatacagatggcccatttgggttaataactcacgcatatgtcgcgcaccaccgccggaagcggcctggtaggttgcaacggacacccaatcaacaagatcattggcgaataaaccccccagcgacatcaacatcaggcttacggtacagttaccgccaacaaaagtcctgataccattatttaatccgtcggtaatgacgtcctgattgacggggtcaagaatgatgatggcgtcatctttcatgcgcagagatgatgctgcgtcaatccagtaaccttgccatccgctttcacgaagctttggatagatttcgttggtataatcgccgccctgacaggtcacaatgatatcgagggcctttagcgcctccagatcaaaggcatcctgaagtgtgccagtggttccgccaaaagacggcgcagcctgaccaagctgagaagtagaaaagaagacagggcgaatggcgtcgaagtcgcgctcttcaaccatgcgttgcatgagaacggagccgaccataccgcgccagccgataaaaccaacatttttcat

SEQ ID NO: 3 - DNA, 1188 bp, Escherichia coli
  source 1..1188: mol_type = genomic DNA
atggcggacaaaaagcttgatactcaactggtgaatgcaggacgcagcaaaaaatacacgctcggtgcggtaaatagcgtgattcagcgcgcgtcttcgctggtctttgacagtgtggaagccaaaaaacacgcgacacgtaatcgcgccaatggcgagttgttctatggacggcgtggaacgttaacccatttctccttacaacaagcgatgtgtgaactggaaggtggcgcaggctgtgtgctatttccctgcggggcggcagcggttgctaattccattcttgcttttgtcgaacagggcgatcatgtgttgatgaccaacaccgcctatgaaccgagtcaggatttctgtagcaaaatcctcagcaaactgggcgtaacgacatcgtggtttgatccgctgattggtgccgatatcgttaatcatctgcagccaaacactaaaatcgtgtttctggaatcgccaggttccatcaccatggaagtccacgatgttccggcgattgttgccgccgtacgcagtgtggtcccggatgccatcattatgatcgacaacacctgggcagccggtgtgctgtttaaggcgctggattttggcatcgatgtttctattcaggccgccaccaaatatctggttgggcattcagatgcgatgattggcactgccgtgtgcaatgcccgttgctgggagcagctgcgagagaatgcctatctgatgggccagatggtcgatgccgataccgcctatataaccagccgtggcctgcgcactttgggggttcgcctgcgtcaacatcatgaaagcagtctgaaagtggctgaatggctggcagaacatccccaagtagcacgagttaaccaccctgctctgcctggcagtaaaggatacgaattctggaaacgagactttacaggcagcagcgggctattttcctttgtgcttaagaaaaaactcaatgatgaagagctggcgaactatctggataacttcagtttattcagcatggcctactcgtggggcgggtatgaatcgttgatcctggcaaatcaaccagaacatatcgccgccattcgcccacaaggcaagatcgattttagcgggaccttgattcgcctgcatattggtctggaagatgtcgacgatctgattgccgatctggacgccggttttgcgcgaattgtataa

SEQ ID NO: 4 - DNA, 1071 bp, Escherichia coli
  source 1..1071: mol_type = genomic DNA
atgacccgtccgatacaggccagcctcgatctgcaggcattaaaacagaatctgtccattgtccgccaggccgcgccgcgcgcgcgcgtctggtcggtggtaaaagcgaacgcttacgggcacggtattgagcgtatctggagcgcgatcggggctaccgatggctttgcattgcttaacctggaagaggcaataacgttacgtgagcgcggctggaaaggaccgatcctgatgctggaaggatttttccatgctcaggatctggagatttatgaccagcaccgcctgaccacctgcgtacacagcaactggcagctcaaagcactgcaaaatgcgcggctaaaagcaccgttggatatttatcttaaagtgaacagtggaatgaatcggttgggcttccagcccgatcgcgtgcttaccgtctggcagcagttgcgggcgatggcgaatgttggcgaaatgaccctgatgtcacattttgccgaagcggaacatcctgatggaatttccggcgcgatggcgcgtattgagcaggcggcggaagggctggagtgtcggcgttcgttgtccaattcggcggcgactctgtggcacccggaagcgcattttgactgggttcggcctggcattattttgtatggcgcttcgccgtccggtcagtggcgtgatatcgccaataccggattacgtccggtgatgacgctaagcagtgagattattggtgtccagacgctaaaagcgggcgagcgtgtgggctacggcggtcgctatactgcgcgcgatgaacagcgaatcggcattgtcgccgcaggatacgccgacggttatccgcgccacgcgcctaccggtacccctgttttagtggacggcgttcgcaccatgacggtggggacagtctcgatggatatgctggcggtcgatttaacgccttgcccgcaagcgggtattggtacgccagttgagctgtggggcaaggagatcaaaattgatgatgtcgccgccgctgccggaacggtaggctatgagttgatgtgcgcgctggcgttacgcgtcccggttgtgacggtgtaa

SEQ ID NO: 5 - DNA, 858 bp, Escherichia coli
  source 1..858: mol_type = genomic DNA
tcagcctaaaactgccagtttttcgagcgtttcgaagccgtaacgctgtaaaacgggcaataattgttcagcttctggcgtcattgccatacaaaaggcaatattcgcatcggcagattttgcatccggggcttcatgttctaacagccaggccgttcggcgagcaatcgctgcgccagaatccaccagccgggttccctctggcagcacctgtaacagttcttcttgtagtagagggaaatgggtacaccccagtacaacggtatctggcggctctttcattcttaaccacgggcgtaggatacgttttagcgcatccagagaaacatcttcgccatgcagcttcgcttcagccaactcaaccatctctgccgagcccagcatttctatctggcattcattagcgaaacgcgcgatcagctcatgagtataagaacgtttaacagttccgcgggttgccagtaatccgacaatgccatttgccgtcagacgtgcagcaggtttaatcgccggcacgacaccaacaaccgggaagtcgaacttttcgcgtaatgcaggaagtgaaacggtactggcggtgttgcaagcgaccacagccagcgcaaggggataacgttcttgcactgcggtgacaatttccaccactcgctcaacaataaacacttcgcttttttcgccatacgggaaagcgacgttatcgaaagcataaatgtaatggagatccggtaagagatgccggatctcgtcatagaccgacaacccaccgacgccggagtcaaacaccagcacggtgggacgtggttcagaaggtgtagctgccagacaaggtgtattcccgtcctgcagtttggtagccat